European Patent Application EP 4 455 287 A1, published October 30, 2024. Title: OPTIMIZED CYP4V2 GENE AND APPLICATION THEREOF. Applicant: Suzhou NGGT Biotechnology Co.,Ltd. The sequence listing filed with the application follows.

SEQUENCE LISTING (28 sequences)

SEQ ID NO: 1 - DNA, 145 bp, synthetic construct
  source 1..145: mol_type = other DNA
ttggccactccctctctgcgcgctcgctcgctcactgaggccgggcgaccaaaggtcgcccgacgcccgggctttgcccgggcggcctcagtgagcgagcgagcgcgcagagagggagtggccaactccatcactaggggttcct

SEQ ID NO: 2 - DNA, 380 bp, synthetic construct
  source 1..380: mol_type = other DNA
gacattgattattgactagttattaatagtaatcaattacggggtcattagttcatagcccatatatggagttccgcgttacataacttacggtaaatggcccgcctggctgaccgcccaacgacccccgcccattgacgtcaataatgacgtatgttcccatagtaacgccaatagggactttccattgacgtcaatgggtggagtatttacggtaaactgcccacttggcagtacatcaagtgtatcatatgccaagtacgccccctattgacgtcaatgacggtaaatggcccgcctggcattatgcccagtacatgaccttatgggactttcctacttggcagtacatctacgtattagtcatcgctattaccatg

SEQ ID NO: 3 - DNA, 278 bp, synthetic construct
  source 1..278: mol_type = other DNA
tcgaggtgagccccacgttctgcttcactctccccatctcccccccctccccacccccaattttgtatttatttattttttaattattttgtgcagcgatgggggcggggggggggggggggcgcgcgccaggcggggcggggcggggcgaggggcggggcggggcgaggcggagaggtgcggcggcagccaatcagagcggcgcgctccgaaagtttccttttatggcgaggcggcggcggcggcggccctataaaaagcgaagcgcgcggcgggcg

SEQ ID NO: 4 - DNA, 1017 bp, synthetic construct
  source 1..1017: mol_type = other DNA
ggagtcgctgcgcgctgccttcgccccgtgccccgctccgccgccgcctcgcgccgcccgccccggctctgactgaccgcgttactcccacaggtgagcgggcgggacggcccttctcctccgggctgtaattagcgcttggtttaatgacggcttgtttcttttctgtggctgcgtgaaagccttgaggggctccgggagggccctttgtgcggggggagcggctcggggggtgcgtgcgtgtgtgtgtgcgtggggagcgccgcgtgcggctccgcgctgcccggcggctgtgagcgctgcgggcgcggcgcggggctttgtgcgctccgcagtgtgcgcgaggggagcgcggccgggggcggtgccccgcggtgcggggggggctgcgaggggaacaaaggctgcgtgcggggtgtgtgcgtgggggggtgagcagggggtgtgggcgcgtcggtcgggctgcaaccccccctgcacccccctccccgagttgctgagcacggcccggcttcgggtgcggggctccgtacggggcgtggcgcggggctcgccgtgccgggcggggggtggcggcaggtgggggtgccgggcggggcggggccgcctcgggccggggagggctcgggggaggggcgcggcggcccccggagcgccggcggctgtcgaggcgcggcgagccgcagccattgccttttatggtaatcgtgcgagagggcgcagggacttcctttgtcccaaatctgtgcggagccgaaatctgggaggcgccgccgcaccccctctagcgggcgcggggcgaagcggtgcggcgccggcaggaaggaaatgggcggggagggccttcgtgcgtcgccgcgccgccgtccccttctccctctccagcctcggggctgtccgcggggggacggctgccttcgggggggacggggcagggcggggttcggcttctggcgtgtgaccggcggctctagagcctctgctaaccatgttcatgccttcttctttttcctacag

SEQ ID NO: 5 - DNA, 1572 bp, synthetic construct
  source 1..1572: mol_type = other DNA
gctggcctgtggctgggcctggtgtggcagaagctgttgctgtggggggctgcctctgccctgagcctggctggggctagcctggtgttgagcctgctgcagagagtggctagctatgctagaaagtggcagcagatgagacccatccccacagtggcaagagcctaccctctggtgggccatgccctgctgatgaagcctgatggcagagagttctttcagcagatcatagagtacacagaggagtacagacacatgcccctgctgaaactgtgggtgggccctgtgcccatggtggctctgtacaatgctgagaatgtggaggtgattctgacaagcagcaagcagattgacaagagctccatgtacaagttcctggagccctggctgggcctgggactgctgacaagcactggcaacaagtggagaagcagaagaaagatgctgacccccaccttccacttcaccatcctggaggacttcctggacattatgaatgagcaagccaacatcctggtgaaaaagctggaaaagcacatcaaccaagaggccttcaactgcttcttctacatcaccctgtgtgccctggacatcatctgtgagacagccatgggcaagaacatcggggcccagagcaatgatgactctgagtatgtgagagctgtgtacagaatgtctgagatgatcttcagaagaatcaagatgccctggctgtggctggacctgtggtacctgatgttcaaggagggctgggagcacaaaaagagcctgcagatcctgcacaccttcaccaactctgtgatcgccgagagagccaatgagatgaatgccaatgaggactgcagaggggatggcagaggctctgcccctagcaagaacaagagaagagccttcctggacctgttgctgtctgtgaccgacgatgagggcaacagactgagccatgaggacatcagagaagaggtggacacatttatgtttgagggccatgacaccacagctgctgccataaactggagcctgtacctgctgggcagcaaccctgaggtgcagaagaaggtggaccatgagctggatgatgtgtttggcaagtctgacagacctgccacagtggaggacctgaagaagctgagatacctggagtgtgtgatcaaggagaccctgagactgttcccctctgtgcccctgtttgctagatctgtgtctgaggactgtgaggtggctggctatagagtgctgaagggcacagaggctgtgatcatcccctatgccctgcacagagaccctagatacttccccaaccctgaggagtttcagcctgagagattcttccctgagaatgcccaaggcagacacccctatgcctatgtgccattctctgctggcccaagaaactgcattgggcagaagtttgctgtgatggaggagaagaccatcctgagctgcatcttgagacacttctggattgagagcaatcagaagagagaggagctgggcctggaggggcagctgatactgagaccaagcaatggcatctggatcaagctgaagagaagaaatgctgatgagaga

SEQ ID NO: 6 - DNA, 1572 bp, synthetic construct
  source 1..1572: mol_type = other DNA
gctggcctgtggctgggcctggtgtggcagaagctgctgctgtggggagctgcctctgccctgtctctggctggagccagcctggtgctgagcctgctgcagagagtggccagctatgccaggaaatggcaacagatgagacctatccccacagtggccagagcctaccccctggttggccatgccctgctgatgaagcctgatggcagagagttcttccagcagatcattgagtacacagaagagtacagacacatgcctctgctgaagctgtgggtgggccctgtgcccatggtggccctgtacaatgcagagaatgtggaagtgatcctgaccagcagcaagcagatagacaagtccagcatgtacaagttcctggaaccttggctgggcctgggcctgctcacctccacaggcaacaagtggagaagcagaaggaagatgctgaccccaaccttccacttcaccatcctggaggactttctggacatcatgaatgagcaggccaacatcctggtcaaaaaactggaaaagcacatcaaccaggaagccttcaactgcttcttctacatcaccctgtgtgccctggacatcatctgcgagacagccatgggcaagaacatcggagcccagagcaatgatgactctgaatatgtcagggcagtgtacagaatgtctgagatgatcttccggcggatcaagatgccttggctgtggctggacctgtggtacctgatgttcaaagagggctgggagcacaagaagagcctgcagatcctgcacaccttcaccaacagcgtgattgctgagcgggccaatgaaatgaacgccaatgaggactgcagaggagatggcagaggctctgcccccagcaagaacaagagaagagccttcctggacctgctgctgtccgtgacagatgatgagggcaacagactgagccacgaggacatcagagaggaagtggacacctttatgtttgaaggccatgacaccacagctgctgccatcaactggagcctgtacctcctgggcagcaaccctgaggtgcagaagaaggtggaccatgagctggatgatgtgtttggcaagtctgacagacctgccacagtggaagacctgaagaaactcaggtacctggaatgtgtgatcaaagagaccctgagactgttcccaagtgtgcctctgtttgccagatctgtctctgaggactgtgaagtggctggctacagagtgctgaagggcacagaggcagttatcatcccctatgccctgcacagagaccccagatacttccccaaccctgaagagttccagcctgagagattcttcccagagaatgcccagggcagacacccttatgcctatgtgcccttctcagctggacctagaaactgcataggccaaaagtttgcagtgatggaagagaagaccatcctgagctgcatcctgaggcacttctggattgagagcaaccagaagagagaggaactgggcctggaaggacagctgatcctgaggcctagcaatggcatctggatcaagctgaaaagaagaaatgctgatgagagg

SEQ ID NO: 7 - DNA, 1572 bp, synthetic construct
  source 1..1572: mol_type = other DNA
gctggcctgtggctgggcctggtgtggcagaaactgctgctgtggggagctgcctctgccctgtctctggctggagcctcccttgtcctgtccctcctgcaaagagttgccagctatgccagaaagtggcagcagatgagacccatccccacagtggccagggcctacccactggtgggccatgccctgctgatgaagcctgatggcagagaattctttcagcagatcatagagtacacagaggagtacagacacatgcctctgctgaagctgtgggtgggccctgtgcctatggtggccctgtacaatgctgagaatgtggaagtgatcctgaccagcagcaagcagattgacaagagcagcatgtacaagttcctggagccttggctgggcctgggcctgctgaccagcacaggcaacaagtggagaagcaggagaaagatgctgacccccaccttccacttcaccatcctggaagacttcctggacatcatgaatgagcaggccaacatcctggtgaaaaagctggaaaaacacatcaaccaggaagccttcaactgcttcttctacattaccctgtgtgccctggacatcatctgcgagacagccatgggaaaaaacatcggagctcagagcaatgatgacagcgagtatgtgagagcagtgtaccggatgagcgaaatgatcttcagacggatcaagatgccctggctgtggctggacctgtggtacctcatgtttaaggagggctgggaacacaagaagagcctgcagatcctgcacaccttcacaaacagtgtgatcgctgaaagggccaacgagatgaatgccaatgaggattgcagaggcgatggccgcggctccgcccctagcaagaacaagagaagagccttcctggacctgctgctgtctgtcaccgatgacgagggcaaccggctgtctcatgaggacatcagagaagaggtggacaccttcatgtttgagggccacgacaccacagccgccgccatcaactggagcctgtacctgcttggcagcaaccctgaggtgcaaaagaaggtggaccatgagctggatgatgtttttggcaaatctgacagacctgccacagtggaggacctgaagaaactgagatacctggagtgtgtgatcaaggaaaccctgagactcttccctagtgtgcctctgtttgccagatctgtctcagaggactgtgaggtggctggctacagagtgctgaagggcacagaagcagtgatcatcccctatgccctgcacagagaccccagatacttccccaaccctgaggaattccagccagagaggttcttccctgagaatgcccagggaagacacccatatgcctatgtgcctttctctgctggccccagaaactgcattggacagaagtttgctgtgatggaggaaaagaccatcctgagctgcatcctgagacacttctggatagaaagcaaccagaagagggaagagctgggcctggaaggccagctgatcctgaggcctagcaatggcatctggatcaaactgaagagaagaaatgcagatgagaga

SEQ ID NO: 8 - DNA, 1572 bp, synthetic construct
  source 1..1572: mol_type = other DNA
gctggcctgtggctgggcctggtgtggcagaagctgctgctgtggggagctgcctctgccctgtccctggctggagcctctctggtgctgagcctgctgcagagagtggccagctatgccaggaaatggcaacagatgagacccatcccaacagtggccagagcctaccccctggttggccatgccctgctgatgaagcctgatggcagagagttcttccagcagatcattgagtacacagaggaatacagacacatgcctctgctgaagctgtgggtgggccctgtgcccatggtggccctgtacaatgcagagaatgtggaagtgatcctgacctccagcaagcagatagacaagagcagcatgtacaagttcctggaaccttggctgggccttggcctgctcaccagcacaggcaacaagtggagaagcagaaggaagatgctgacccctaccttccacttcaccatcctggaggactttctggacatcatgaatgagcaggccaacatcctggtcaaaaagctggaaaagcacatcaaccaggaggccttcaactgcttcttctacatcaccctgtgtgccctggacatcatctgcgagacagccatgggcaaaaacatcggagcccagagcaatgatgactctgagtatgtgcgggctgtgtaccggatgagcgaaatgatcttcagacggatcaagatgccctggctgtggctggacctctggtacctgatgttcaaagaaggctgggagcacaagaagagcctgcagatcctgcacaccttcaccaacagcgtgattgcagaaagagccaatgagatgaatgccaacgaggactgcagaggagatggcagaggctctgcccctagcaagaacaagagaagggcctttctggacctgctgctgtctgtcacagatgatgagggcaacagactgagccacgaggacatcagagaggaagtggacaccttcatgtttgaaggccatgacaccacagctgctgccatcaactggtccctgtacctgctgggcagcaaccctgaggtgcagaagaaggtggaccatgagctggatgatgtgtttggcaagtctgacagacctgccacagtggaagacctgaaaaagctgagatacctggaatgtgtgatcaaagagaccctgagactgttcccttctgtgcctctgtttgccagaagtgtttctgaggactgtgaagtggctggctacagagtgctgaagggcacagaggcagtcatcatcccctatgccctgcacagagaccccaggtacttccccaaccctgaggagttccagcctgaaagattcttcccagagaatgcccagggcagacacccatatgcctatgtgcccttctcagctggacctagaaactgcataggacaaaagtttgcagtgatggaagagaagaccatcctgagctgcatcctgaggcacttctggattgagagcaaccagaaaagagaggaactgggcctggaaggccagctgatcctcaggcctagcaatggcatctggatcaagctgaagagaaggaatgctgatgagaga

SEQ ID NO: 9 - DNA, 1572 bp, synthetic construct
  source 1..1572: mol_type = other DNA
gcggggctctggctggggctcgtgtggcagaagctgctgctgtggggcgcggcgagtgccctttccctggccggcgccagtctggtcctgagcctgctgcagagggtggcgagctacgcgcggaaatggcagcagatgcggcccatccccacggtggcccgcgcctacccactggtgggccacgcgctgctgatgaagccggacgggcgagaattttttcagcagatcattgagtacacagaggaataccgccacatgccgctgctgaagctctgggtcgggccagtgcccatggtggccctttataatgcagaaaatgtggaggtaattttaactagttcaaagcaaattgacaaatcctctatgtacaagtttttagaaccatggcttggcctaggacttcttacaagtactggaaacaaatggcgctccaggagaaagatgttaacacccactttccattttaccattctggaagatttcttagatatcatgaatgaacaagcaaatatattggttaagaaacttgaaaaacacattaaccaagaagcatttaactgctttttttacatcactctttgtgccttagatatcatctgtgaaacagctatggggaagaatattggtgctcaaagtaatgatgattccgagtatgtccgtgcagtttatagaatgagtgagatgatatttcgaagaataaagatgccctggctttggcttgatctctggtaccttatgtttaaagaaggatgggaacacaaaaagagccttcagatcctacatacttttaccaacagtgtcatcgctgaacgggccaatgaaatgaacgccaatgaagactgtagaggtgatggcaggggctctgccccctccaaaaataaacgcagggcctttcttgacttgcttttaagtgtgactgatgacgaagggaacaggctaagtcatgaagatattcgagaagaagttgacaccttcatgtttgaggggcacgatacaactgcagctgcaataaactggtccttatacctgttgggttctaacccagaagtccagaaaaaagtggatcatgaattggatgacgtgtttgggaagtctgaccgtcccgctacagtagaagacctgaagaaacttcggtatctggaatgtgttattaaggagacccttcgcctttttccttctgttcctttatttgcccgtagtgttagtgaagattgtgaagtggcaggttacagagttctaaaaggcactgaagccgtcatcattccctatgcattgcacagagatccgagatacttccccaaccccgaggagttccagcctgagcggttcttccccgagaatgcacaagggcgccatccatatgcctacgtgcccttctctgctggccccaggaactgtataggtcaaaagtttgctgtgatggaagaaaagaccattctttcgtgcatcctgaggcacttttggatagaatccaaccagaaaagagaagagcttggtctagaaggacagttgattcttcgtccaagtaatggcatctggatcaagttgaagaggagaaatgcagatgaacgc

SEQ ID NO: 10 - DNA, 225 bp, synthetic construct
  source 1..225: mol_type = other DNA
ctgtgccttctagttgccagccatctgttgtttgcccctcccccgtgccttccttgaccctggaaggtgccactcccactgtcctttcctaataaaatgaggaaattgcatcgcattgtctgagtaggtgtcattctattctggggggtggggtggggcaggacagcaagggggaggattgggaagacaatagcaggcatgctggggatgcggtgggctctatgg

SEQ ID NO: 11 - DNA, 145 bp, synthetic construct
  source 1..145: mol_type = other DNA
aggaacccctagtgatggagttggccactccctctctgcgcgctcgctcgctcactgaggccgggcgaccaaaggtcgcccgacgcccgggctttgcccgggcggcctcagtgagcgagcgagcgcgcagagagggagtggccaa

SEQ ID NO: 12 - DNA, 3961 bp, synthetic construct
  source 1..3961: mol_type = other DNA
ttggccactccctctctgcgcgctcgctcgctcactgaggccgggcgaccaaaggtcgcccgacgcccgggctttgcccgggcggcctcagtgagcgagcgagcgcgcagagagggagtggccaactccatcactaggggttcctctcgaggagcttggcccattgcatacgttgtatccatatcataatatgtacatttatattggctcatgtccaacattaccgccatgttactagtgtcgacattgattattgactagttattaatagtaatcaattacggggtcattagttcatagcccatatatggagttccgcgttacataacttacggtaaatggcccgcctggctgaccgcccaacgacccccgcccattgacgtcaataatgacgtatgttcccatagtaacgccaatagggactttccattgacgtcaatgggtggagtatttacggtaaactgcccacttggcagtacatcaagtgtatcatatgccaagtacgccccctattgacgtcaatgacggtaaatggcccgcctggcattatgcccagtacatgaccttatgggactttcctacttggcagtacatctacgtattagtcatcgctattaccatggtcgaggtgagccccacgttctgcttcactctccccatctcccccccctccccacccccaattttgtatttatttattttttaattattttgtgcagcgatgggggcggggggggggggggggcgcgcgccaggcggggcggggcggggcgaggggcggggcggggcgaggcggagaggtgcggcggcagccaatcagagcggcgcgctccgaaagtttccttttatggcgaggcggcggcggcggcggccctataaaaagcgaagcgcgcggcgggcgggagtcgctgcgcgctgccttcgccccgtgccccgctccgccgccgcctcgcgccgcccgccccggctctgactgaccgcgttactcccacaggtgagcgggcgggacggcccttctcctccgggctgtaattagcgcttggtttaatgacggcttgtttcttttctgtggctgcgtgaaagccttgaggggctccgggagggccctttgtgcggggggagcggctcggggggtgcgtgcgtgtgtgtgtgcgtggggagcgccgcgtgcggctccgcgctgcccggcggctgtgagcgctgcgggcgcggcgcggggctttgtgcgctccgcagtgtgcgcgaggggagcgcggccgggggcggtgccccgcggtgcggggggggctgcgaggggaacaaaggctgcgtgcggggtgtgtgcgtgggggggtgagcagggggtgtgggcgcgtcggtcgggctgcaaccccccctgcacccccctccccgagttgctgagcacggcccggcttcgggtgcggggctccgtacggggcgtggcgcggggctcgccgtgccgggcggggggtggcggcaggtgggggtgccgggcggggcggggccgcctcgggccggggagggctcgggggaggggcgcggcggcccccggagcgccggcggctgtcgaggcgcggcgagccgcagccattgccttttatggtaatcgtgcgagagggcgcagggacttcctttgtcccaaatctgtgcggagccgaaatctgggaggcgccgccgcaccccctctagcgggcgcggggcgaagcggtgcggcgccggcaggaaggaaatgggcggggagggccttcgtgcgtcgccgcgccgccgtccccttctccctctccagcctcggggctgtccgcggggggacggctgccttcgggggggacggggcagggcggggttcggcttctggcgtgtgaccggcggctctagagcctctgctaaccatgttcatgccttcttctttttcctacagctcctgggcaacgtgctggttattgtgctgtctcatcattttggcaaagaattcggcgcgccgccaccatggctggcctgtggctgggcctggtgtggcagaagctgctgctgtggggagctgcctctgccctgtccctggctggagcctctctggtgctgagcctgctgcagagagtggccagctatgccaggaaatggcaacagatgagacccatcccaacagtggccagagcctaccccctggttggccatgccctgctgatgaagcctgatggcagagagttcttccagcagatcattgagtacacagaggaatacagacacatgcctctgctgaagctgtgggtgggccctgtgcccatggtggccctgtacaatgcagagaatgtggaagtgatcctgacctccagcaagcagatagacaagagcagcatgtacaagttcctggaaccttggctgggccttggcctgctcaccagcacaggcaacaagtggagaagcagaaggaagatgctgacccctaccttccacttcaccatcctggaggactttctggacatcatgaatgagcaggccaacatcctggtcaaaaagctggaaaagcacatcaaccaggaggccttcaactgcttcttctacatcaccctgtgtgccctggacatcatctgcgagacagccatgggcaaaaacatcggagcccagagcaatgatgactctgagtatgtgcgggctgtgtaccggatgagcgaaatgatcttcagacggatcaagatgccctggctgtggctggacctctggtacctgatgttcaaagaaggctgggagcacaagaagagcctgcagatcctgcacaccttcaccaacagcgtgattgcagaaagagccaatgagatgaatgccaacgaggactgcagaggagatggcagaggctctgcccctagcaagaacaagagaagggcctttctggacctgctgctgtctgtcacagatgatgagggcaacagactgagccacgaggacatcagagaggaagtggacaccttcatgtttgaaggccatgacaccacagctgctgccatcaactggtccctgtacctgctgggcagcaaccctgaggtgcagaagaaggtggaccatgagctggatgatgtgtttggcaagtctgacagacctgccacagtggaagacctgaaaaagctgagatacctggaatgtgtgatcaaagagaccctgagactgttcccttctgtgcctctgtttgccagaagtgtttctgaggactgtgaagtggctggctacagagtgctgaagggcacagaggcagtcatcatcccctatgccctgcacagagaccccaggtacttccccaaccctgaggagttccagcctgaaagattcttcccagagaatgcccagggcagacacccatatgcctatgtgcccttctcagctggacctagaaactgcataggacaaaagtttgcagtgatggaagagaagaccatcctgagctgcatcctgaggcacttctggattgagagcaaccagaaaagagaggaactgggcctggaaggccagctgatcctcaggcctagcaatggcatctggatcaagctgaagagaaggaatgctgatgagagataaagatctgcctcgactgtgccttctagttgccagccatctgttgtttgcccctcccccgtgccttccttgaccctggaaggtgccactcccactgtcctttcctaataaaatgaggaaattgcatcgcattgtctgagtaggtgtcattctattctggggggtggggtggggcaggacagcaagggggaggattgggaagacaatagcaggcatgctggggatgcggtgggctctatggatcccctaactacaaggaacccctagtgatggagttggccactccctctctgcgcgctcgctcgctcactgaggccgggcgaccaaaggtcgcccgacgcccgggctttgcccgggcggcctcagtgagcgagcgagcgcgcagagagggagtggccaa

SEQ ID NO: 13 - DNA, 3961 bp, synthetic construct
  source 1..3961: mol_type = other DNA
ttggccactccctctctgcgcgctcgctcgctcactgaggccgggcgaccaaaggtcgcccgacgcccgggctttgcccgggcggcctcagtgagcgagcgagcgcgcagagagggagtggccaactccatcactaggggttcctctcgaggagcttggcccattgcatacgttgtatccatatcataatatgtacatttatattggctcatgtccaacattaccgccatgttactagtgtcgacattgattattgactagttattaatagtaatcaattacggggtcattagttcatagcccatatatggagttccgcgttacataacttacggtaaatggcccgcctggctgaccgcccaacgacccccgcccattgacgtcaataatgacgtatgttcccatagtaacgccaatagggactttccattgacgtcaatgggtggagtatttacggtaaactgcccacttggcagtacatcaagtgtatcatatgccaagtacgccccctattgacgtcaatgacggtaaatggcccgcctggcattatgcccagtacatgaccttatgggactttcctacttggcagtacatctacgtattagtcatcgctattaccatggtcgaggtgagccccacgttctgcttcactctccccatctcccccccctccccacccccaattttgtatttatttattttttaattattttgtgcagcgatgggggcggggggggggggggggcgcgcgccaggcggggcggggcggggcgaggggcggggcggggcgaggcggagaggtgcggcggcagccaatcagagcggcgcgctccgaaagtttccttttatggcgaggcggcggcggcggcggccctataaaaagcgaagcgcgcggcgggcgggagtcgctgcgcgctgccttcgccccgtgccccgctccgccgccgcctcgcgccgcccgccccggctctgactgaccgcgttactcccacaggtgagcgggcgggacggcccttctcctccgggctgtaattagcgcttggtttaatgacggcttgtttcttttctgtggctgcgtgaaagccttgaggggctccgggagggccctttgtgcggggggagcggctcggggggtgcgtgcgtgtgtgtgtgcgtggggagcgccgcgtgcggctccgcgctgcccggcggctgtgagcgctgcgggcgcggcgcggggctttgtgcgctccgcagtgtgcgcgaggggagcgcggccgggggcggtgccccgcggtgcggggggggctgcgaggggaacaaaggctgcgtgcggggtgtgtgcgtgggggggtgagcagggggtgtgggcgcgtcggtcgggctgcaaccccccctgcacccccctccccgagttgctgagcacggcccggcttcgggtgcggggctccgtacggggcgtggcgcggggctcgccgtgccgggcggggggtggcggcaggtgggggtgccgggcggggcggggccgcctcgggccggggagggctcgggggaggggcgcggcggcccccggagcgccggcggctgtcgaggcgcggcgagccgcagccattgccttttatggtaatcgtgcgagagggcgcagggacttcctttgtcccaaatctgtgcggagccgaaatctgggaggcgccgccgcaccccctctagcgggcgcggggcgaagcggtgcggcgccggcaggaaggaaatgggcggggagggccttcgtgcgtcgccgcgccgccgtccccttctccctctccagcctcggggctgtccgcggggggacggctgccttcgggggggacggggcagggcggggttcggcttctggcgtgtgaccggcggctctagagcctctgctaaccatgttcatgccttcttctttttcctacagctcctgggcaacgtgctggttattgtgctgtctcatcattttggcaaagaattcggcgcgccgccaccatggctggcctgtggctgggcctggtgtggcagaagctgctgctgtggggagctgcctctgccctgtctctggctggagccagcctggtgctgagcctgctgcagagagtggccagctatgccaggaaatggcaacagatgagacctatccccacagtggccagagcctaccccctggttggccatgccctgctgatgaagcctgatggcagagagttcttccagcagatcattgagtacacagaagagtacagacacatgcctctgctgaagctgtgggtgggccctgtgcccatggtggccctgtacaatgcagagaatgtggaagtgatcctgaccagcagcaagcagatagacaagtccagcatgtacaagttcctggaaccttggctgggcctgggcctgctcacctccacaggcaacaagtggagaagcagaaggaagatgctgaccccaaccttccacttcaccatcctggaggactttctggacatcatgaatgagcaggccaacatcctggtcaaaaaactggaaaagcacatcaaccaggaagccttcaactgcttcttctacatcaccctgtgtgccctggacatcatctgcgagacagccatgggcaagaacatcggagcccagagcaatgatgactctgaatatgtcagggcagtgtacagaatgtctgagatgatcttccggcggatcaagatgccttggctgtggctggacctgtggtacctgatgttcaaagagggctgggagcacaagaagagcctgcagatcctgcacaccttcaccaacagcgtgattgctgagcgggccaatgaaatgaacgccaatgaggactgcagaggagatggcagaggctctgcccccagcaagaacaagagaagagccttcctggacctgctgctgtccgtgacagatgatgagggcaacagactgagccacgaggacatcagagaggaagtggacacctttatgtttgaaggccatgacaccacagctgctgccatcaactggagcctgtacctcctgggcagcaaccctgaggtgcagaagaaggtggaccatgagctggatgatgtgtttggcaagtctgacagacctgccacagtggaagacctgaagaaactcaggtacctggaatgtgtgatcaaagagaccctgagactgttcccaagtgtgcctctgtttgccagatctgtctctgaggactgtgaagtggctggctacagagtgctgaagggcacagaggcagttatcatcccctatgccctgcacagagaccccagatacttccccaaccctgaagagttccagcctgagagattcttcccagagaatgcccagggcagacacccttatgcctatgtgcccttctcagctggacctagaaactgcataggccaaaagtttgcagtgatggaagagaagaccatcctgagctgcatcctgaggcacttctggattgagagcaaccagaagagagaggaactgggcctggaaggacagctgatcctgaggcctagcaatggcatctggatcaagctgaaaagaagaaatgctgatgagaggtaaagatctgcctcgactgtgccttctagttgccagccatctgttgtttgcccctcccccgtgccttccttgaccctggaaggtgccactcccactgtcctttcctaataaaatgaggaaattgcatcgcattgtctgagtaggtgtcattctattctggggggtggggtggggcaggacagcaagggggaggattgggaagacaatagcaggcatgctggggatgcggtgggctctatggatcccctaactacaaggaacccctagtgatggagttggccactccctctctgcgcgctcgctcgctcactgaggccgggcgaccaaaggtcgcccgacgcccgggctttgcccgggcggcctcagtgagcgagcgagcgcgcagagagggagtggccaa

SEQ ID NO: 14 - DNA, 3961 bp, synthetic construct
  source 1..3961: mol_type = other DNA
ttggccactccctctctgcgcgctcgctcgctcactgaggccgggcgaccaaaggtcgcccgacgcccgggctttgcccgggcggcctcagtgagcgagcgagcgcgcagagagggagtggccaactccatcactaggggttcctctcgaggagcttggcccattgcatacgttgtatccatatcataatatgtacatttatattggctcatgtccaacattaccgccatgttactagtgtcgacattgattattgactagttattaatagtaatcaattacggggtcattagttcatagcccatatatggagttccgcgttacataacttacggtaaatggcccgcctggctgaccgcccaacgacccccgcccattgacgtcaataatgacgtatgttcccatagtaacgccaatagggactttccattgacgtcaatgggtggagtatttacggtaaactgcccacttggcagtacatcaagtgtatcatatgccaagtacgccccctattgacgtcaatgacggtaaatggcccgcctggcattatgcccagtacatgaccttatgggactttcctacttggcagtacatctacgtattagtcatcgctattaccatggtcgaggtgagccccacgttctgcttcactctccccatctcccccccctccccacccccaattttgtatttatttattttttaattattttgtgcagcgatgggggcggggggggggggggggcgcgcgccaggcggggcggggcggggcgaggggcggggcggggcgaggcggagaggtgcggcggcagccaatcagagcggcgcgctccgaaagtttccttttatggcgaggcggcggcggcggcggccctataaaaagcgaagcgcgcggcgggcgggagtcgctgcgcgctgccttcgccccgtgccccgctccgccgccgcctcgcgccgcccgccccggctctgactgaccgcgttactcccacaggtgagcgggcgggacggcccttctcctccgggctgtaattagcgcttggtttaatgacggcttgtttcttttctgtggctgcgtgaaagccttgaggggctccgggagggccctttgtgcggggggagcggctcggggggtgcgtgcgtgtgtgtgtgcgtggggagcgccgcgtgcggctccgcgctgcccggcggctgtgagcgctgcgggcgcggcgcggggctttgtgcgctccgcagtgtgcgcgaggggagcgcggccgggggcggtgccccgcggtgcggggggggctgcgaggggaacaaaggctgcgtgcggggtgtgtgcgtgggggggtgagcagggggtgtgggcgcgtcggtcgggctgcaaccccccctgcacccccctccccgagttgctgagcacggcccggcttcgggtgcggggctccgtacggggcgtggcgcggggctcgccgtgccgggcggggggtggcggcaggtgggggtgccgggcggggcggggccgcctcgggccggggagggctcgggggaggggcgcggcggcccccggagcgccggcggctgtcgaggcgcggcgagccgcagccattgccttttatggtaatcgtgcgagagggcgcagggacttcctttgtcccaaatctgtgcggagccgaaatctgggaggcgccgccgcaccccctctagcgggcgcggggcgaagcggtgcggcgccggcaggaaggaaatgggcggggagggccttcgtgcgtcgccgcgccgccgtccccttctccctctccagcctcggggctgtccgcggggggacggctgccttcgggggggacggggcagggcggggttcggcttctggcgtgtgaccggcggctctagagcctctgctaaccatgttcatgccttcttctttttcctacagctcctgggcaacgtgctggttattgtgctgtctcatcattttggcaaagaattcggcgcgccgccaccatggctggcctgtggctgggcctggtgtggcagaaactgctgctgtggggagctgcctctgccctgtctctggctggagcctcccttgtcctgtccctcctgcaaagagttgccagctatgccagaaagtggcagcagatgagacccatccccacagtggccagggcctacccactggtgggccatgccctgctgatgaagcctgatggcagagaattctttcagcagatcatagagtacacagaggagtacagacacatgcctctgctgaagctgtgggtgggccctgtgcctatggtggccctgtacaatgctgagaatgtggaagtgatcctgaccagcagcaagcagattgacaagagcagcatgtacaagttcctggagccttggctgggcctgggcctgctgaccagcacaggcaacaagtggagaagcaggagaaagatgctgacccccaccttccacttcaccatcctggaagacttcctggacatcatgaatgagcaggccaacatcctggtgaaaaagctggaaaaacacatcaaccaggaagccttcaactgcttcttctacattaccctgtgtgccctggacatcatctgcgagacagccatgggaaaaaacatcggagctcagagcaatgatgacagcgagtatgtgagagcagtgtaccggatgagcgaaatgatcttcagacggatcaagatgccctggctgtggctggacctgtggtacctcatgtttaaggagggctgggaacacaagaagagcctgcagatcctgcacaccttcacaaacagtgtgatcgctgaaagggccaacgagatgaatgccaatgaggattgcagaggcgatggccgcggctccgcccctagcaagaacaagagaagagccttcctggacctgctgctgtctgtcaccgatgacgagggcaaccggctgtctcatgaggacatcagagaagaggtggacaccttcatgtttgagggccacgacaccacagccgccgccatcaactggagcctgtacctgcttggcagcaaccctgaggtgcaaaagaaggtggaccatgagctggatgatgtttttggcaaatctgacagacctgccacagtggaggacctgaagaaactgagatacctggagtgtgtgatcaaggaaaccctgagactcttccctagtgtgcctctgtttgccagatctgtctcagaggactgtgaggtggctggctacagagtgctgaagggcacagaagcagtgatcatcccctatgccctgcacagagaccccagatacttccccaaccctgaggaattccagccagagaggttcttccctgagaatgcccagggaagacacccatatgcctatgtgcctttctctgctggccccagaaactgcattggacagaagtttgctgtgatggaggaaaagaccatcctgagctgcatcctgagacacttctggatagaaagcaaccagaagagggaagagctgggcctggaaggccagctgatcctgaggcctagcaatggcatctggatcaaactgaagagaagaaatgcagatgagagataaagatctgcctcgactgtgccttctagttgccagccatctgttgtttgcccctcccccgtgccttccttgaccctggaaggtgccactcccactgtcctttcctaataaaatgaggaaattgcatcgcattgtctgagtaggtgtcattctattctggggggtggggtggggcaggacagcaagggggaggattgggaagacaatagcaggcatgctggggatgcggtgggctctatggatcccctaactacaaggaacccctagtgatggagttggccactccctctctgcgcgctcgctcgctcactgaggccgggcgaccaaaggtcgcccgacgcccgggctttgcccgggcggcctcagtgagcgagcgagcgcgcagagagggagtggccaa

SEQ ID NO: 15 - DNA, 3961 bp, synthetic construct
  source 1..3961: mol_type = other DNA
ttggccactccctctctgcgcgctcgctcgctcactgaggccgggcgaccaaaggtcgcccgacgcccgggctttgcccgggcggcctcagtgagcgagcgagcgcgcagagagggagtggccaactccatcactaggggttcctctcgaggagcttggcccattgcatacgttgtatccatatcataatatgtacatttatattggctcatgtccaacattaccgccatgttactagtgtcgacattgattattgactagttattaatagtaatcaattacggggtcattagttcatagcccatatatggagttccgcgttacataacttacggtaaatggcccgcctggctgaccgcccaacgacccccgcccattgacgtcaataatgacgtatgttcccatagtaacgccaatagggactttccattgacgtcaatgggtggagtatttacggtaaactgcccacttggcagtacatcaagtgtatcatatgccaagtacgccccctattgacgtcaatgacggtaaatggcccgcctggcattatgcccagtacatgaccttatgggactttcctacttggcagtacatctacgtattagtcatcgctattaccatggtcgaggtgagccccacgttctgcttcactctccccatctcccccccctccccacccccaattttgtatttatttattttttaattattttgtgcagcgatgggggcggggggggggggggggcgcgcgccaggcggggcggggcggggcgaggggcggggcggggcgaggcggagaggtgcggcggcagccaatcagagcggcgcgctccgaaagtttccttttatggcgaggcggcggcggcggcggccctataaaaagcgaagcgcgcggcgggcgggagtcgctgcgcgctgccttcgccccgtgccccgctccgccgccgcctcgcgccgcccgccccggctctgactgaccgcgttactcccacaggtgagcgggcgggacggcccttctcctccgggctgtaattagcgcttggtttaatgacggcttgtttcttttctgtggctgcgtgaaagccttgaggggctccgggagggccctttgtgcggggggagcggctcggggggtgcgtgcgtgtgtgtgtgcgtggggagcgccgcgtgcggctccgcgctgcccggcggctgtgagcgctgcgggcgcggcgcggggctttgtgcgctccgcagtgtgcgcgaggggagcgcggccgggggcggtgccccgcggtgcggggggggctgcgaggggaacaaaggctgcgtgcggggtgtgtgcgtgggggggtgagcagggggtgtgggcgcgtcggtcgggctgcaaccccccctgcacccccctccccgagttgctgagcacggcccggcttcgggtgcggggctccgtacggggcgtggcgcggggctcgccgtgccgggcggggggtggcggcaggtgggggtgccgggcggggcggggccgcctcgggccggggagggctcgggggaggggcgcggcggcccccggagcgccggcggctgtcgaggcgcggcgagccgcagccattgccttttatggtaatcgtgcgagagggcgcagggacttcctttgtcccaaatctgtgcggagccgaaatctgggaggcgccgccgcaccccctctagcgggcgcggggcgaagcggtgcggcgccggcaggaaggaaatgggcggggagggccttcgtgcgtcgccgcgccgccgtccccttctccctctccagcctcggggctgtccgcggggggacggctgccttcgggggggacggggcagggcggggttcggcttctggcgtgtgaccggcggctctagagcctctgctaaccatgttcatgccttcttctttttcctacagctcctgggcaacgtgctggttattgtgctgtctcatcattttggcaaagaattcggcgcgccgccaccatggctggcctgtggctgggcctggtgtggcagaagctgttgctgtggggggctgcctctgccctgagcctggctggggctagcctggtgttgagcctgctgcagagagtggctagctatgctagaaagtggcagcagatgagacccatccccacagtggcaagagcctaccctctggtgggccatgccctgctgatgaagcctgatggcagagagttctttcagcagatcatagagtacacagaggagtacagacacatgcccctgctgaaactgtgggtgggccctgtgcccatggtggctctgtacaatgctgagaatgtggaggtgattctgacaagcagcaagcagattgacaagagctccatgtacaagttcctggagccctggctgggcctgggactgctgacaagcactggcaacaagtggagaagcagaagaaagatgctgacccccaccttccacttcaccatcctggaggacttcctggacattatgaatgagcaagccaacatcctggtgaaaaagctggaaaagcacatcaaccaagaggccttcaactgcttcttctacatcaccctgtgtgccctggacatcatctgtgagacagccatgggcaagaacatcggggcccagagcaatgatgactctgagtatgtgagagctgtgtacagaatgtctgagatgatcttcagaagaatcaagatgccctggctgtggctggacctgtggtacctgatgttcaaggagggctgggagcacaaaaagagcctgcagatcctgcacaccttcaccaactctgtgatcgccgagagagccaatgagatgaatgccaatgaggactgcagaggggatggcagaggctctgcccctagcaagaacaagagaagagccttcctggacctgttgctgtctgtgaccgacgatgagggcaacagactgagccatgaggacatcagagaagaggtggacacatttatgtttgagggccatgacaccacagctgctgccataaactggagcctgtacctgctgggcagcaaccctgaggtgcagaagaaggtggaccatgagctggatgatgtgtttggcaagtctgacagacctgccacagtggaggacctgaagaagctgagatacctggagtgtgtgatcaaggagaccctgagactgttcccctctgtgcccctgtttgctagatctgtgtctgaggactgtgaggtggctggctatagagtgctgaagggcacagaggctgtgatcatcccctatgccctgcacagagaccctagatacttccccaaccctgaggagtttcagcctgagagattcttccctgagaatgcccaaggcagacacccctatgcctatgtgccattctctgctggcccaagaaactgcattgggcagaagtttgctgtgatggaggagaagaccatcctgagctgcatcttgagacacttctggattgagagcaatcagaagagagaggagctgggcctggaggggcagctgatactgagaccaagcaatggcatctggatcaagctgaagagaagaaatgctgatgagagataaagatctgcctcgactgtgccttctagttgccagccatctgttgtttgcccctcccccgtgccttccttgaccctggaaggtgccactcccactgtcctttcctaataaaatgaggaaattgcatcgcattgtctgagtaggtgtcattctattctggggggtggggtggggcaggacagcaagggggaggattgggaagacaatagcaggcatgctggggatgcggtgggctctatggatcccctaactacaaggaacccctagtgatggagttggccactccctctctgcgcgctcgctcgctcactgaggccgggcgaccaaaggtcgcccgacgcccgggctttgcccgggcggcctcagtgagcgagcgagcgcgcagagagggagtggccaa

SEQ ID NO: 16 - DNA, 3961 bp, synthetic construct
  source 1..3961: mol_type = other DNA
ttggccactccctctctgcgcgctcgctcgctcactgaggccgggcgaccaaaggtcgcccgacgcccgggctttgcccgggcggcctcagtgagcgagcgagcgcgcagagagggagtggccaactccatcactaggggttcctctcgaggagcttggcccattgcatacgttgtatccatatcataatatgtacatttatattggctcatgtccaacattaccgccatgttactagtgtcgacattgattattgactagttattaatagtaatcaattacggggtcattagttcatagcccatatatggagttccgcgttacataacttacggtaaatggcccgcctggctgaccgcccaacgacccccgcccattgacgtcaataatgacgtatgttcccatagtaacgccaatagggactttccattgacgtcaatgggtggagtatttacggtaaactgcccacttggcagtacatcaagtgtatcatatgccaagtacgccccctattgacgtcaatgacggtaaatggcccgcctggcattatgcccagtacatgaccttatgggactttcctacttggcagtacatctacgtattagtcatcgctattaccatggtcgaggtgagccccacgttctgcttcactctccccatctcccccccctccccacccccaattttgtatttatttattttttaattattttgtgcagcgatgggggcggggggggggggggggcgcgcgccaggcggggcggggcggggcgaggggcggggcggggcgaggcggagaggtgcggcggcagccaatcagagcggcgcgctccgaaagtttccttttatggcgaggcggcggcggcggcggccctataaaaagcgaagcgcgcggcgggcgggagtcgctgcgcgctgccttcgccccgtgccccgctccgccgccgcctcgcgccgcccgccccggctctgactgaccgcgttactcccacaggtgagcgggcgggacggcccttctcctccgggctgtaattagcgcttggtttaatgacggcttgtttcttttctgtggctgcgtgaaagccttgaggggctccgggagggccctttgtgcggggggagcggctcggggggtgcgtgcgtgtgtgtgtgcgtggggagcgccgcgtgcggctccgcgctgcccggcggctgtgagcgctgcgggcgcggcgcggggctttgtgcgctccgcagtgtgcgcgaggggagcgcggccgggggcggtgccccgcggtgcggggggggctgcgaggggaacaaaggctgcgtgcggggtgtgtgcgtgggggggtgagcagggggtgtgggcgcgtcggtcgggctgcaaccccccctgcacccccctccccgagttgctgagcacggcccggcttcgggtgcggggctccgtacggggcgtggcgcggggctcgccgtgccgggcggggggtggcggcaggtgggggtgccgggcggggcggggccgcctcgggccggggagggctcgggggaggggcgcggcggcccccggagcgccggcggctgtcgaggcgcggcgagccgcagccattgccttttatggtaatcgtgcgagagggcgcagggacttcctttgtcccaaatctgtgcggagccgaaatctgggaggcgccgccgcaccccctctagcgggcgcggggcgaagcggtgcggcgccggcaggaaggaaatgggcggggagggccttcgtgcgtcgccgcgccgccgtccccttctccctctccagcctcggggctgtccgcggggggacggctgccttcgggggggacggggcagggcggggttcggcttctggcgtgtgaccggcggctctagagcctctgctaaccatgttcatgccttcttctttttcctacagctcctgggcaacgtgctggttattgtgctgtctcatcattttggcaaagaattcggcgcgccgccaccatggcggggctctggctggggctcgtgtggcagaagctgctgctgtggggcgcggcgagtgccctttccctggccggcgccagtctggtcctgagcctgctgcagagggtggcgagctacgcgcggaaatggcagcagatgcggcccatccccacggtggcccgcgcctacccactggtgggccacgcgctgctgatgaagccggacgggcgagaattttttcagcagatcattgagtacacagaggaataccgccacatgccgctgctgaagctctgggtcgggccagtgcccatggtggccctttataatgcagaaaatgtggaggtaattttaactagttcaaagcaaattgacaaatcctctatgtacaagtttttagaaccatggcttggcctaggacttcttacaagtactggaaacaaatggcgctccaggagaaagatgttaacacccactttccattttaccattctggaagatttcttagatatcatgaatgaacaagcaaatatattggttaagaaacttgaaaaacacattaaccaagaagcatttaactgctttttttacatcactctttgtgccttagatatcatctgtgaaacagctatggggaagaatattggtgctcaaagtaatgatgattccgagtatgtccgtgcagtttatagaatgagtgagatgatatttcgaagaataaagatgccctggctttggcttgatctctggtaccttatgtttaaagaaggatgggaacacaaaaagagccttcagatcctacatacttttaccaacagtgtcatcgctgaacgggccaatgaaatgaacgccaatgaagactgtagaggtgatggcaggggctctgccccctccaaaaataaacgcagggcctttcttgacttgcttttaagtgtgactgatgacgaagggaacaggctaagtcatgaagatattcgagaagaagttgacaccttcatgtttgaggggcacgatacaactgcagctgcaataaactggtccttatacctgttgggttctaacccagaagtccagaaaaaagtggatcatgaattggatgacgtgtttgggaagtctgaccgtcccgctacagtagaagacctgaagaaacttcggtatctggaatgtgttattaaggagacccttcgcctttttccttctgttcctttatttgcccgtagtgttagtgaagattgtgaagtggcaggttacagagttctaaaaggcactgaagccgtcatcattccctatgcattgcacagagatccgagatacttccccaaccccgaggagttccagcctgagcggttcttccccgagaatgcacaagggcgccatccatatgcctacgtgcccttctctgctggccccaggaactgtataggtcaaaagtttgctgtgatggaagaaaagaccattctttcgtgcatcctgaggcacttttggatagaatccaaccagaaaagagaagagcttggtctagaaggacagttgattcttcgtccaagtaatggcatctggatcaagttgaagaggagaaatgcagatgaacgctaaagatctgcctcgactgtgccttctagttgccagccatctgttgtttgcccctcccccgtgccttccttgaccctggaaggtgccactcccactgtcctttcctaataaaatgaggaaattgcatcgcattgtctgagtaggtgtcattctattctggggggtggggtggggcaggacagcaagggggaggattgggaagacaatagcaggcatgctggggatgcggtgggctctatggatcccctaactacaaggaacccctagtgatggagttggccactccctctctgcgcgctcgctcgctcactgaggccgggcgaccaaaggtcgcccgacgcccgggctttgcccgggcggcctcagtgagcgagcgagcgcgcagagagggagtggccaa

SEQ ID NO: 17 - skipped

SEQ ID NO: 18 - DNA, 23 bp, synthetic construct
  source 1..23: mol_type = other DNA
agtatgtccgtgcagtttatagg

SEQ ID NO: 19 - DNA, 23 bp, synthetic construct
  source 1..23: mol_type = other DNA
catacaggtcatcgctgaacggg

SEQ ID NO: 20 - DNA, 23 bp, synthetic construct
  source 1..23: mol_type = other DNA
tcatacaggtcatcgctgaacgg

SEQ ID NO: 21 - DNA, 23 bp, synthetic construct
  source 1..23: mol_type = other DNA
gattatcattcaaatcatacagg

SEQ ID NO: 22 - DNA, 20 bp, synthetic construct
  source 1..20: mol_type = other DNA
gaaatcacactccaccggga

SEQ ID NO: 23 - DNA, 24 bp, synthetic construct
  source 1..24: mol_type = other DNA
acctttactgcttaaacacatgct

SEQ ID NO: 24 - DNA, 20 bp, synthetic construct
  source 1..20: mol_type = other DNA
caggcagcagaaatcgcaag

SEQ ID NO: 25 - DNA, 20 bp, synthetic construct
  source 1..20: mol_type = other DNA
agcctgttcccttcgtcatc

SEQ ID NO: 26 - DNA, 102 bp, synthetic construct
  source 1..102: mol_type = other DNA
taactagggtgcatccaagtccaaacagaagcatgtgattatcattcaaagcgaacgggccaatgaaatgaacgccaatgaagactgtagaggtgatggcag

SEQ ID NO: 27 - protein, 525 aa, synthetic construct
MAGLWLGLVWQKLLLWGAASALSLAGASLVLSLLQRVASYARKWQQMRPIPTVARAYPLVGHALLMKPDGREFFQQIIEYTEEYRHMPLLKLWVGPVPMVALYNAENVEVILTSSKQIDKSSMYKFLEPWLGLGLLTSTGNKWRSRRKMLTPTFHFTILEDFLDIMNEQANILVKKLEKHINQEAFNCFFYITLCALDIICETAMGKNIGAQSNDDSEYVRAVYRMSEMIFRRIKMPWLWLDLWYLMFKEGWEHKKSLQILHTFTNSVIAERANEMNANEDCRGDGRGSAPSKNKRRAFLDLLLSVTDDEGNRLSHEDIREEVDTFMFEGHDTTAAAINWSLYLLGSNPEVQKKVDHELDDVFGKSDRPATVEDLKKLRYLECVIKETLRLFPSVPLFARSVSEDCEVAGYRVLKGTEAVIIPYALHRDPRYFPNPEEFQPERFFPENAQGRHPYAYVPFSAGPRNCIGQKFAVMEEKTILSCILRHFWIESNQKREELGLEGQLILRPSNGIWIKLKRRNADER

SEQ ID NO: 28 - DNA, 1575 bp, synthetic construct
  source 1..1575: mol_type = other DNA
atggcggggctctggctggggctcgtgtggcagaagctgctgctgtggggcgcggcgagtgccctttccctggccggcgccagtctggtcctgagcctgctgcagagggtggcgagctacgcgcggaaatggcagcagatgcggcccatccccacggtggcccgcgcctacccactggtgggccacgcgctgctgatgaagccggacgggcgagaattttttcagcagatcattgagtacacagaggaataccgccacatgccgctgctgaagctctgggtcgggccagtgcccatggtggccctttataatgcagaaaatgtggaggtaattttaactagttcaaagcaaattgacaaatcctctatgtacaagtttttagaaccatggcttggcctaggacttcttacaagtactggaaacaaatggcgctccaggagaaagatgttaacacccactttccattttaccattctggaagatttcttagatatcatgaatgaacaagcaaatatattggttaagaaacttgaaaaacacattaaccaagaagcatttaactgctttttttacatcactctttgtgccttagatatcatctgtgaaacagctatggggaagaatattggtgctcaaagtaatgatgattccgagtatgtccgtgcagtttatagaatgagtgagatgatatttcgaagaataaagatgccctggctttggcttgatctctggtaccttatgtttaaagaaggatgggaacacaaaaagagccttcagatcctacatacttttaccaacagtgtcatcgctgaacgggccaatgaaatgaacgccaatgaagactgtagaggtgatggcaggggctctgccccctccaaaaataaacgcagggcctttcttgacttgcttttaagtgtgactgatgacgaagggaacaggctaagtcatgaagatattcgagaagaagttgacaccttcatgtttgaggggcacgatacaactgcagctgcaataaactggtccttatacctgttgggttctaacccagaagtccagaaaaaagtggatcatgaattggatgacgtgtttgggaagtctgaccgtcccgctacagtagaagacctgaagaaacttcggtatctggaatgtgttattaaggagacccttcgcctttttccttctgttcctttatttgcccgtagtgttagtgaagattgtgaagtggcaggttacagagttctaaaaggcactgaagccgtcatcattccctatgcattgcacagagatccgagatacttccccaaccccgaggagttccagcctgagcggttcttccccgagaatgcacaagggcgccatccatatgcctacgtgcccttctctgctggccccaggaactgtataggtcaaaagtttgctgtgatggaagaaaagaccattctttcgtgcatcctgaggcacttttggatagaatccaaccagaaaagagaagagcttggtctagaaggacagttgattcttcgtccaagtaatggcatctggatcaagttgaagaggagaaatgcagatgaacgc